European Patent Application EP 4 252 854 A2, published October 4, 2023. Title: Humanized antibody specific for CD22 and chimeric antigen receptor using the same. Applicant: InnoBation Bio Co., Ltd. Application EP. The sequence listing filed with the application follows.

SEQUENCE LISTING (55 sequences)

SEQ ID NO: 1 - protein, 9 aa, synthetic construct
GFSLTSYDI

SEQ ID NO: 2 - protein, 7 aa, synthetic construct
IWTGGGT

SEQ ID NO: 3 - protein, 12 aa, synthetic construct
VPHYYGYAMDYW

SEQ ID NO: 4 - protein, 6 aa, synthetic construct
QDINKY

SEQ ID NO: 5 - skipped

SEQ ID NO: 6 - protein, 8 aa, synthetic construct
LQYDNLLT

SEQ ID NO: 7 - protein, 117 aa, synthetic construct
EVQLQESGPGLVAPSQSLSITCTVSGFSLTSYDISWIRQPPGKGLEWLGVIWTGGGTNYNSAFMSRLSISKDNSKSQVFLKMNSLQTDDTAIYYCVPHYYGYAMDYWGQGTSVTVSS

SEQ ID NO: 8 - protein, 106 aa, synthetic construct
DIVLTQSPSSLSASLGGKVTITCKASQDINKYIAWYQHKPGKGPRLLIHYTSTLQPGIPSRFSGSGSGRDYSFSISNLEPEDIATYYCLQYDNLLTFGAGTKLELK

SEQ ID NO: 9 - DNA, 351 bp, synthetic construct
  source 1..351: mol_type = other DNA
gaggtgcagctgcaggagtcaggacctggcctggtggcgccctcacagagcctgtccattacctgcactgtctctgggttctcattaaccagctatgatataagctggattcgccagccaccaggaaagggtctggagtggcttggagtaatatggactggtggaggcacaaattataattcagctttcatgtccagactgagcatcagcaaggacaactccaagagccaagttttcttaaaaatgaacagtctgcaaactgatgacacagccatatattactgtgtccctcattactacggctatgctatggactactggggtcaaggaacctcagtcaccgtctcctca

SEQ ID NO: 10 - DNA, 318 bp, synthetic construct
  source 1..318: mol_type = other DNA
gatattgtgctgacccagtctccatcctcactgtctgcatctctgggaggcaaagtcaccatcacttgcaaggcaagccaagacattaacaagtatatagcttggtaccaacacaagcctggaaaaggtcctaggctgctcatacattacacatctacattacagccaggcatcccatcaaggttcagtggaagtgggtctgggagagattattccttcagcatcagcaacctggagcctgaagatattgcaacttattattgtctacagtatgataatctgctcacgttcggtgctgggaccaagctggagctgaaa

SEQ ID NO: 11 - protein, 117 aa, synthetic construct
EVQLQESGPGLVKPSQTLSLTCTVSGFSLTSYDISWIRQPPGKGLEWLGVIWTGGGTNYNSALKSRVTISKDNSKSQVSLKLSSVTAADTAVYYCVPHYYGYAMDYWGQGTTVTVSS

SEQ ID NO: 12 - protein, 106 aa, synthetic construct
EIVLTQSPATLSLSPGERATLSCRASQDINKYIAWYQQKPGQAPRLLIHYTSTRQTGIPARFSGSGSGRDYTLTISSLEPEDFAVYYCLQYDNLLTFGGGTKLEIK

SEQ ID NO: 13 - DNA, 351 bp, synthetic construct
  source 1..351: mol_type = other DNA
gaggtgcagctgcaggagagcggccccggcctggtgaagccgagccagactctttctctgacctgcaccgtgtccggcttctctcttacgagctacgacatctcgtggatccggcagccgcctgggaaaggcttagagtggctaggggtgatttggaccggcgggggtaccaactacaactccgcgctcaaatcccgcgtcactatttctaaggacaattccaagagccaggtctcgctgaagctctcgtccgtgaccgccgcggacaccgcagtttattactgcgtgcctcattactacggctacgccatggattattggggccagggcaccacagtaacagtcagctcc

SEQ ID NO: 14 - DNA, 318 bp, synthetic construct
  source 1..318: mol_type = other DNA
gagatcgtgctgactcagagcccggccacccttagcctgagtccaggcgagcgcgctacgttgtcatgccgagcttcccaggacattaacaagtacatcgcgtggtaccagcagaagcccggacaggccccccgcctgctcatccactacacctccacccgccagactggcatccctgccaggttttcaggctccggttctggccgtgactacaccctgaccatctctagtttggagcccgaagatttcgccgtgtactactgtctgcaatatgacaacctgctgaccttcggagggggtaccaagctggagatcaag

SEQ ID NO: 15 - protein, 117 aa, synthetic construct
EVQLKESGPVLVKPTETLTLTCTVSGFSLTSYDISWIRQPPGKALEWLGVIWTGGGTNYNSALKSRLTISKDNSKSQVVLTMTNMDPVDTATYYCVPHYYGYAMDYWGQGTTVTVSS

SEQ ID NO: 16 - protein, 106 aa, synthetic construct; identical to SEQ ID NO: 12

SEQ ID NO: 17 - DNA, 351 bp, synthetic construct
  source 1..351: mol_type = other DNA
gaggtgcagctgaaggagagcgggccggtgctggtgaagcctaccgagactctgaccctgacctgcactgtttccggcttctctctgacgagctacgacatcagttggatccgccagccacccggcaaagcgttggaatggctcggggtaatttggaccggtggcgggaccaactacaacagcgcgctcaaatcgcggctaaccatctcaaaggacaactccaagtcccaagtggtgttaactatgacaaatatggatccggtcgacaccgctacctattactgcgtgcctcattactacggctacgccatggattattggggccagggcacgaccgtgaccgtctccagt

SEQ ID NO: 18 - DNA, 318 bp, synthetic construct
  source 1..318: mol_type = other DNA
gagatcgtgttgacccagagccctgccacgctgagcctgtcccccggggagcgcgccactctttcgtgtagggcttcccaggacattaacaagtacatcgcatggtaccagcagaagcccggacaggccccccgcctgctcatccactacacatccacccgccagacaggcatcccggctcgattctctggttctggcagcggtcgtgattacacccttactatttcttccctggagccagaggactttgcggtgtactactgcctgcagtatgacaacctgctgaccttcggcggaggcaccaagctggagatcaag

SEQ ID NO: 19 - protein, 15 aa, synthetic construct
GGGGSGGGGSGGGGS

SEQ ID NO: 20 - DNA, 45 bp, synthetic construct
  source 1..45: mol_type = other DNA
ggcggaggcggcagcggcggaggcggctctggcggcggcgggagc

SEQ ID NO: 21 - DNA, 45 bp, synthetic construct
  source 1..45: mol_type = other DNA
gggggcggcggatctggtggtggaggctccggcggtggcggttcc

SEQ ID NO: 22 - DNA, 45 bp, synthetic construct
  source 1..45: mol_type = other DNA
ggcggcggtggctccggtggaggcggatctggcggtggcgggtcg

SEQ ID NO: 23 - protein, 238 aa, synthetic construct
DIVLTQSPSSLSASLGGKVTITCKASQDINKYIAWYQHKPGKGPRLLIHYTSTLQPGIPSRFSGSGSGRDYSFSISNLEPEDIATYYCLQYDNLLTFGAGTKLELKGGGGSGGGGSGGGGSEVQLQESGPGLVAPSQSLSITCTVSGFSLTSYDISWIRQPPGKGLEWLGVIWTGGGTNYNSAFMSRLSISKDNSKSQVFLKMNSLQTDDTAIYYCVPHYYGYAMDYWGQGTSVTVSS

SEQ ID NO: 24 - DNA, 714 bp, synthetic construct
  source 1..714: mol_type = other DNA
gatatcgtgctgacccagagcccttctagcctgagcgcctctctgggcggcaaggtgaccatcacctgcaaggccagccaggacatcaacaagtacatcgcctggtaccagcacaagcctggaaaaggccctagactgctgatccactacaccagcacactccagcctggcatccccagcagattcagcggatctggaagcggcagagattacagcttcagcatttctaatctggaacctgaggacatcgctacatactattgtctgcagtacgacaacctgctgaccttcggcgctggcaccaagctggagctgaaaggcggaggcggcagcggcggaggcggctctggcggcggcgggagcgaggtgcagctgcaggagagcggccccggactggtcgccccaagccaatctctgtccatcacatgcaccgtgtccggctttagcctgacatcatatgatatcagctggatccggcagccacctggcaagggcctggaatggctgggcgttatctggaccggcggaggcacaaactacaactccgccttcatgagccggctgagcatctctaaggacaatagcaagtcccaggtgttcctgaagatgaacagcctgcaaacagacgacaccgccatctactactgcgtgccccactactacggctacgccatggactactggggccagggcaccagcgtgaccgtgtccagc

SEQ ID NO: 25 - protein, 238 aa, synthetic construct
EIVLTQSPATLSLSPGERATLSCRASQDINKYIAWYQQKPGQAPRLLIHYTSTRQTGIPARFSGSGSGRDYTLTISSLEPEDFAVYYCLQYDNLLTFGGGTKLEIKGGGGSGGGGSGGGGSEVQLQESGPGLVKPSQTLSLTCTVSGFSLTSYDISWIRQPPGKGLEWLGVIWTGGGTNYNSALKSRVTISKDNSKSQVSLKLSSVTAADTAVYYCVPHYYGYAMDYWGQGTTVTVSS

SEQ ID NO: 26 - DNA, 714 bp, synthetic construct
  source 1..714: mol_type = other DNA
gagatcgtgctgactcagagcccggccacccttagcctgagtccaggcgagcgcgctacgttgtcatgccgagcttcccaggacattaacaagtacatcgcgtggtaccagcagaagcccggacaggccccccgcctgctcatccactacacctccacccgccagactggcatccctgccaggttttcaggctccggttctggccgtgactacaccctgaccatctctagtttggagcccgaagatttcgccgtgtactactgtctgcaatatgacaacctgctgaccttcggagggggtaccaagctggagatcaaggggggcggcggatctggtggtggaggctccggcggtggcggttccgaggtgcagctgcaggagagcggccccggcctggtgaagccgagccagactctttctctgacctgcaccgtgtccggcttctctcttacgagctacgacatctcgtggatccggcagccgcctgggaaaggcttagagtggctaggggtgatttggaccggcgggggtaccaactacaactccgcgctcaaatcccgcgtcactatttctaaggacaattccaagagccaggtctcgctgaagctctcgtccgtgaccgccgcggacaccgcagtttattactgcgtgcctcattactacggctacgccatggattattggggccagggcaccacagtaacagtcagctcc

SEQ ID NO: 27 - protein, 238 aa, synthetic construct
EIVLTQSPATLSLSPGERATLSCRASQDINKYIAWYQQKPGQAPRLLIHYTSTRQTGIPARFSGSGSGRDYTLTISSLEPEDFAVYYCLQYDNLLTFGGGTKLEIKGGGGSGGGGSGGGGSEVQLKESGPVLVKPTETLTLTCTVSGFSLTSYDISWIRQPPGKALEWLGVIWTGGGTNYNSALKSRLTISKDNSKSQVVLTMTNMDPVDTATYYCVPHYYGYAMDYWGQGTTVTVSS

SEQ ID NO: 28 - DNA, 714 bp, synthetic construct
  source 1..714: mol_type = other DNA
gagatcgtgttgacccagagccctgccacgctgagcctgtcccccggggagcgcgccactctttcgtgtagggcttcccaggacattaacaagtacatcgcatggtaccagcagaagcccggacaggccccccgcctgctcatccactacacatccacccgccagacaggcatcccggctcgattctctggttctggcagcggtcgtgattacacccttactatttcttccctggagccagaggactttgcggtgtactactgcctgcagtatgacaacctgctgaccttcggcggaggcaccaagctggagatcaagggcggcggtggctccggtggaggcggatctggcggtggcgggtcggaggtgcagctgaaggagagcgggccggtgctggtgaagcctaccgagactctgaccctgacctgcactgtttccggcttctctctgacgagctacgacatcagttggatccgccagccacccggcaaagcgttggaatggctcggggtaatttggaccggtggcgggaccaactacaacagcgcgctcaaatcgcggctaaccatctcaaaggacaactccaagtcccaagtggtgttaactatgacaaatatggatccggtcgacaccgctacctattactgcgtgcctcattactacggctacgccatggattattggggccagggcacgaccgtgaccgtctccagt

SEQ ID NO: 29 - DNA, 1178 bp, synthetic construct
  source 1..1178: mol_type = other DNA
gctccggtgcccgtcagtgggcagagcgcacatcgcccacagtccccgagaagttggggggaggggtcggcaattgaaccggtgcctagagaaggtggcgcggggtaaactgggaaagtgatgtcgtgtactggctccgcctttttcccgagggtgggggagaaccgtatataagtgcagtagtcgccgtgaacgttctttttcgcaacgggtttgccgccagaacacaggtaagtgccgtgtgtggttcccgcgggcctggcctctttacgggttatggcccttgcgtgccttgaattacttccacctggctgcagtacgtgattcttgatcccgagcttcgggttggaagtgggtgggagagttcgaggccttgcgcttaaggagccccttcgcctcgtgcttgagttgaggcctggcctgggcgctggggccgccgcgtgcgaatctggtggcaccttcgcgcctgtctcgctgctttcgataagtctctagccatttaaaatttttgatgacctgctgcgacgctttttttctggcaagatagtcttgtaaatgcgggccaagatctgcacactggtatttcggtttttggggccgcgggcggcgacggggcccgtgcgtcccagcgcacatgttcggcgaggcggggcctgcgagcgcggccaccgagaatcggacgggggtagtctcaagctggccggcctgctctggtgcctggcctcgcgccgccgtgtatcgccccgccctgggcggcaaggctggcccggtcggcaccagttgcgtgagcggaaagatggccgcttcccggccctgctgcagggagctcaaaatggaggacgcggcgctcgggagagcgggcgggtgagtcacccacacaaaggaaaagggcctttccgtcctcagccgtcgcttcatgtgactccactgagtaccgggcgccgtccaggcacctcgattagttctcgagcttttggagtacgtcgtctttaggttggggggaggggttttatgcgatggagtttccccacactgagtgggtggagactgaagttaggccagcttggcacttgatgtaattctccttggaatttgccctttttgagtttggatcttggttcattctcaagcctcagacagtggttcaaagtttttttcttccatttcaggtgtcgtga

SEQ ID NO: 30 - DNA, 63 bp, synthetic construct
  source 1..63: mol_type = other DNA
atggccttaccagtgaccgccttgctcctgccgctggccttgctgctccacgccgccaggccg

SEQ ID NO: 31 - DNA, 135 bp, synthetic construct
  source 1..135: mol_type = other DNA
accacgacgccagcgccgcgaccaccaacaccggcgcccaccatcgcgtcgcagcccctgtccctgcgcccagaggcgtgccggccagcggcggggggcgcagtgcacacgagggggctggacttcgcctgtgat

SEQ ID NO: 32 - DNA, 72 bp, synthetic construct
  source 1..72: mol_type = other DNA
atctacatctgggcgcccttggccgggacttgtggggtccttctcctgtcactggttatcaccctttactgc

SEQ ID NO: 33 - DNA, 126 bp, synthetic construct
  source 1..126: mol_type = other DNA
aaacggggcagaaagaaactcctgtatatattcaaacaaccatttatgagaccagtacaaactactcaagaggaagatggctgtagctgccgatttccagaagaagaagaaggaggatgtgaactg

SEQ ID NO: 34 - DNA, 336 bp, synthetic construct
  source 1..336: mol_type = other DNA
agagtgaagttcagcaggagcgcagacgcccccgcgtacaagcagggccagaaccagctctataacgagctcaatctaggacgaagagaggagtacgatgttttggacaagagacgtggccgggaccctgagatggggggaaagccgagaaggaagaaccctcaggaaggcctgtacaatgaactgcagaaagataagatggcggaggcctacagtgagattgggatgaaaggcgagcgccggaggggcaaggggcacgatggcctttaccagggtctcagtacagccaccaaggacacctacgacgcccttcacatgcaggccctgccccctcgc

SEQ ID NO: 35 - DNA, 591 bp, synthetic construct
  source 1..591: mol_type = other DNA
atcaacctctggattacaaaatttgtgaaagattgactggtattcttaactatgttgctccttttacgctatgtggatacgctgctttaatgcctttgtatcatgctattgcttcccgtatggctttcattttctcctccttgtataaatcctggttgctgtctctttatgaggagttgtggcccgttgtcaggcaacgtggcgtggtgtgcactgtgtttgctgacgcaacccccactggttggggcattgccaccacctgtcagctcctttccgggactttcgctttccccctccctattgccacggcggaactcatcgccgcctgccttgcccgctgctggacaggggctcggctgttgggcactgacaattccgtggtgttgtcggggaagctgacgtcctttccatggctgctcgcctgtgttgccacctggattctgcgcgggacgtccttctgctacgtcccttcggccctcaatccagcggaccttccttcccgcggcctgctgccggctctgcggcctcttccgcgtcttcgccttcgccctcagacgagtcggatctccctttgggccgcctccccgcctg

SEQ ID NO: 36 - protein, 21 aa, synthetic construct
MALPVTALLLPLALLLHAARP

SEQ ID NO: 37 - protein, 45 aa, synthetic construct
TTTPAPRPPTPAPTIASQPLSLRPEACRPAAGGAVHTRGLDFACD

SEQ ID NO: 38 - protein, 24 aa, synthetic construct
IYIWAPLAGTCGVLLLSLVITLYC

SEQ ID NO: 39 - protein, 42 aa, synthetic construct
KRGRKKLLYIFKQPFMRPVQTTQEEDGCSCRFPEEEEGGCEL

SEQ ID NO: 40 - protein, 112 aa, synthetic construct
RVKFSRSADAPAYKQGQNQLYNELNLGRREEYDVLDKRRGRDPEMGGKPRRKNPQEGLYNELQKDKMAEAYSEIGMKGERRRGKGHDGLYQGLSTATKDTYDALHMQALPPR

SEQ ID NO: 41 - protein, 8 aa, synthetic construct
GVSLPDYG

SEQ ID NO: 42 - protein, 7 aa, synthetic construct
IWGSETT

SEQ ID NO: 43 - protein, 14 aa, synthetic construct
AKHYYYGGSYAMDY

SEQ ID NO: 44 - protein, 6 aa, synthetic construct
QDISKY

SEQ ID NO: 45 - skipped

SEQ ID NO: 46 - protein, 9 aa, synthetic construct
QQGNTLPYT

SEQ ID NO: 47 - protein, 119 aa, synthetic construct
EVKLQESGPGLVAPSQSLSVTCTVSGVSLPDYGVSWIRQPPRKGLEWLGVIWGSETTYYNSALKSRLTIIKDNSKSQVFLKMNSLQTDDTAIYYCAKHYYYGGSYAMDYWGQGTSVTVS

SEQ ID NO: 48 - protein, 128 aa, synthetic construct
MALPVTALLLPLALLLHAARPDIQMTQTTSSLSASLGDRVTISCRASQDISKYLNWYQQKPDGTVKLLIYHTSRLHSGVPSRFSGSGSGTDYSLTISNLEQEDIATYFCQQGNTLPYTFGGGTKLEIT

SEQ ID NO: 49 - DNA, 360 bp, synthetic construct
  source 1..360: mol_type = other DNA
tctgaggtgaaactgcaggagtcaggacctggcctggtggcgccctcacagagcctgtccgtcacatgcactgtctcaggggtctcattacccgactatggtgtaagctggattcgccagcctccacgaaagggtctggagtggctgggagtaatatggggtagtgaaaccacatactataattcagctctcaaatccagactgaccatcatcaaggacaactccaagagccaagttttcttaaaaatgaacagtctgcaaactgatgacacagccatttactactgtgccaaacattattactacggtggtagctatgctatggactactggggccaaggaacctcagtcaccgtctcc

SEQ ID NO: 50 - DNA, 384 bp, synthetic construct
  source 1..384: mol_type = other DNA
atggccttaccagtgaccgccttgctcctgccgctggccttgctgctccacgccgccaggccggacatccagatgacacagactacatcctccctgtctgcctctctgggagacagagtcaccatcagttgcagggcaagtcaggacattagtaaatatttaaattggtatcagcagaaaccagatggaactgttaaactcctgatctaccatacatcaagattacactcaggagtcccatcaaggttcagtggcagtgggtctggaacagattattctctcaccattagcaacctggagcaagaagatattgccacttacttttgccaacagggtaatacgcttccgtacacgttcggaggggggaccaagctggagatcaca

SEQ ID NO: 51 - protein, 5 aa, synthetic construct
GGGGS

SEQ ID NO: 52 - DNA, 15 bp, synthetic construct
  source 1..15: mol_type = other DNA
ggcgggggaggctct

SEQ ID NO: 53 - DNA, 15 bp, synthetic construct
  source 1..15: mol_type = other DNA
ggcggagggggctcc

SEQ ID NO: 54 - protein, 18 aa, synthetic construct
GSTSGSGKPGSGEGSTKG

SEQ ID NO: 55 - DNA, 54 bp, synthetic construct
  source 1..54: mol_type = other DNA
ggctccaccagtggttctgggaaacctggtagtggggagggctcgacgaagggg